European Patent Specification EP 3 622 810 B1, published January 3, 2024. Title: METHODS AND COMPOSITIONS FOR EXTENDING SHELF LIFE OF PLANT PRODUCTS. Applicant: Seminis Vegetable Seeds, Inc. The sequence listing filed with the application follows.

SEQUENCE LISTING (32 sequences)

SEQ ID NO: 1 - DNA, 189 bp, Artificial sequence
  Synthetic oligonucleotide
gataggagaaacgtcttattaggtctcggaggtctttacggcgccgccgccacttttgggtcaaactcattggcgtatgcagctccgattatggcaccggacctcacaaaatgtggtccggctgacttaccccaaggggctgtacctacaaactgttgccctccatacaccacaaagattcacgatttc

SEQ ID NO: 2 - DNA, 225 bp, Artificial sequence
  Synthetic oligonucleotide
gagaaaatttgtggcaaattaatcgatgatccaaatttcgcaatccctttttggaactgggatgcacctgatggcatgaagatccctgatatttacacgaataagaaatctccgttgtacgatgctcttcgtgatgcgaagcatcaaccaccgtctctgattgatcttgactacaatggtgacgatgaaaatcttagccgatcgaaacaaacctccacaaatctc

SEQ ID NO: 3 - DNA, 225 bp, Artificial sequence
  Synthetic oligonucleotide
ggagataggaaccagcaaaatggtgaagacatgggtaacttttattctgcagccagagaccctattttctatgcacatcatgcgaatatcgacagaatgtggtcagtttggaaaactctaggaggaagaaggaatgattttacagataaagactggcttgattcttcgttcttgttctacgatgagaacgctgaaatggttcgagtcaaggtgagggattgtctc

SEQ ID NO: 4 - DNA, 226 bp, Artificial sequence
  Synthetic oligonucleotide
gagagatgagtttgcgaagtttgatgtgtttgtgaacgatgaagatgacgggatgagggccacggctgataagacggagttcgccggaagttttgttaatgtccctcataagcataagcatgggaagaatgtgaagacaagattgaggttaggaataagtgagcttttggaggatttgggagctgaagatgatgacaacgtgttggtgacattggtgccgaaaaac

SEQ ID NO: 5 - DNA, 25 bp, Artificial sequence
  Synthetic oligonucleotide
atcgtcaccattgtagtcaagatca

SEQ ID NO: 6 - DNA, 25 bp, Artificial sequence
  Synthetic oligonucleotide
atatcagggatcttcatgccatcag

SEQ ID NO: 7 - RNA, 25 nt, Artificial sequence
  Synthetic oligonucleotide
aucgucaccauuguagucaagauca

SEQ ID NO: 8 - RNA, 25 nt, Artificial sequence
  Synthetic oligonucleotide
auaucagggaucuucaugccaucag

SEQ ID NO: 9 - DNA, 1922 bp, Lactuca sativa
atggcatctcttgcacaatcaccaaccaccaccaccaccaccggtggacggtgcttctcctcctcctccacgtactcttcttccttctctttcaaatcatctcaagttcccatagcacgaatcacgaaccatcgccatgcagtttcatgcaaaggcgccctagatgatgatgaccatcaccatgaaaactcaggcaaatttgataggagaaacgtcttattaggtctcggaggtctttacggcgccgccgccacttttgggtcaaactcattggcgtatgcagctccgattatggcaccggacctcacaaaatgtggtccggctgacttaccccaaggggctgtacctacaaactgttgccctccatacaccacaaagattcacgatttcaaacttccaccaccgtcaaccaccttccgagtccgtccggcagctcatttggctaataaagattacatagccaagttcaataaagccatcgagctcatgaaagctctcccagatgacgatcctcgtagtttcaagcaacaagctgctgttcattgtgcgtattgcgatggggcatacgatcaagtcggtttccctgatctcgagcttcaagtccatggctcatggttgttcttacctttccaccgctattacttatacttcttcgagaaaatttgtggcaaattaatcgatgatccaaatttcgcaatccctttttggaactgggatgcacctgatggcatgaagatccctgatatttacacgaataagaaatctccgttgtacgatgctcttcgtgatgcgaagcatcaaccaccgtctctgattgatcttgactacaatggtgacgatgaaaatcttagccgatcgaaacaaacctccacaaatctcacaattatgtacagacaaatggtgtctagttccaagactgctagtcttttcatgggtagtccttatcgtgcaggtgatgaggctagccctggctctggctcgctcgagagcataccacatggcccggttcatatctggaccggagataggaaccagcaaaatggtgaagacatgggtaacttttattctgcagccagagaccctattttctatgcacatcatgcgaatatcgacagaatgtggtcagtttggaaaactctaggaggaagaaggaatgattttacagataaagactggcttgattcttcgttcttgttctacgatgagaacgctgaaatggttcgagtcaaggtgagggattgtctcgactccaagaagcttgggtacgtttatcaggatgtagagataccatggctaaaaagcaaacccgaaccacgtctgaaaagggctttgagcaagatcaagaagctcgctgtagctcgagccgatgaacacataccctttgcaaaagatgtttttccggcgagtcttgataaggtgataaaagtgctggttccaaggccgaagaaatcaaggagcaagaaacagaaagaggatgaagaagaaattttggtgatagaaggaattgaactgaagagagatgagtttgcgaagtttgatgtgtttgtgaacgatgaagatgacgggatgagggccacggctgataagacggagttcgccggaagttttgttaatgtccctcataagcataagcatgggaagaatgtgaagacaagattgaggttaggaataagtgagcttttggaggatttgggagctgaagatgatgacaacgtgttggtgacattggtgccgaaaaacaaaggtggtgaagtttccattaaagggattaaaatcgagcatgaggattgataaaaataacttttcattttcttgaaaaataaaaaactatgattttgagttgtttcggtaaatatgttgtcgcttggttaatgtatcatcaataaaaataaatttcgaaatcaaagttggatttgaacccc

SEQ ID NO: 10 - DNA, 1001 bp, Artificial sequence
  Synthetic oligonucleotide
aaaagtaaaaataagtttttaaagtattcgtatttatattttaagaaatattagtcaaatataatgaatttttttttatccaaattcaaaaaaacaaatgatatagtttttcgtaatattattttaatgagtttttaaaagaaatctttcaaaagtattattgttaaggatactcacattttgtttaagtgattataagtttttattaaaaaataaataaaacgtgaaaattttcgttctttaaatgaaaaacctttttaatggtttactaaatattatatattatgagctttttgaaatttaataaggttatttagatacaaaattttattttaaaagattacaagctttgaaaataaaaataaatatgatattattcaaaatgattcaaaatatttatgattaaaaaaattatgattaaacatatttatgatttttaattgtttatgatctaaaaatatcataatctaaatattatgatccttaattacataatttatgattcaaaattaaatgtttttataatgatctaaaatttgttattaacaaaaaatttatttaagtgaatatattattatccaaaattatatgattaaaatatattataatctaaaatactacaattgattgtttaatgctccaaaattatatcatccaaaaatagtaaatagtatgatatgaaaacataatgattcctaatatcttatgattcaaaacgtttataaattttaaacatcaaaacctcaaacaaatatttagtttaaaaaaacaaaagaaaatctaaataataaaacaaaaacaaaaaacacaaataacttcaaagatatactaaaatgctatatgaagtggtatgagtttcttacccgtgtgatgacatggaatgtaagtcatgcgtcagttaggaggaacaatcagtggcggagctagaagttttcatttggggcgccgaaaatagaatttgtataaaaattgaagaacagaggggccaaagtcaaacttta

SEQ ID NO: 11 - DNA, 1001 bp, Lactuca sativa
aaaaccaaaattcacaaaatcatttatcacattcgaatacaaaaactaccaacactaaatatttatatttaatttcaaagtatcgaaaatcaaatgacatgttaaaagtatcaaaagtcggtggcttggtaaaagtgtcaatgtcttaggtaggtgggttgcttttttggcaaactttccgtattttgttatacatcttatcctttcttgtcttttggcctcagtttctttacaataaactgcagatatgaaaacaaaagaataaacaaattacaaatgtcaaacgctataatattaataataaggtaaattttttgaagtttgatgcttaaagaggagaaacgttggaagtaaaacttgtaatacagagaaatgaaagttgttataaaaatgaaagtatgatgctataatagaactatatttacaccaagttcaaagtacgacactgtaattagaaaaaggtaaaaatgtacacaaaataaacaaatggaagtgcatcaatcaaatcaacttgagttctaccttatgtacacatatcaaatgacagtttatggtgccaatctacagctaattagcaccggatgcacaagtgactaagaaaattttggtattaatggttttaatcctatgtatgttgtaagaaagatttatatgaaaacatattgcattttttaaaaggtagaaatatgtaacacccggattttcaactaccgattaaatgacaaataatcgttccaacatctcccatgatcaattctaaacttacgtatagactacactacaacggaagcaaaattaaataaaataaaatcttcaattgaagaactttaggtgttacatctttacggaactcctttatcgtcttgttatacaatccctctccttgccttcttactgccacttgctaaatagtttcctgggttgcgcacatataaagtttctatatgggtaagcctaaggcctagtgagttcgtgttgcacatacatgtccatcagttaac

SEQ ID NO: 12 - DNA, 21 bp, Artificial sequence
  Synthetic oligonucleotide
cgtcgagattctgcgagaaag

SEQ ID NO: 13 - DNA, 21 bp, Artificial sequence
  Synthetic oligonucleotide
gcaaacgtcgtcgatgtaagc

SEQ ID NO: 14 - DNA, 30 bp, Artificial sequence
  Synthetic oligonucleotide
ctcctccgtgttgttgatcgtgaatacgtc

SEQ ID NO: 15 - DNA, 22 bp, Artificial sequence
  Synthetic oligonucleotide
gcaagttcaataaagccatcga

SEQ ID NO: 16 - DNA, 22 bp, Artificial sequence
  Synthetic oligonucleotide
cgcaataggcacaatgaacatt

SEQ ID NO: 17 - DNA, 29 bp, Artificial sequence
  Synthetic oligonucleotide
cccagatgacgatcctcgtagctttaagc

SEQ ID NO: 18 - DNA, 23 bp, Artificial sequence
  Synthetic oligonucleotide
aaggcttccagaaacatcaagaa

SEQ ID NO: 19 - DNA, 21 bp, Artificial sequence
  Synthetic oligonucleotide
agactcgccggaaaaacatct

SEQ ID NO: 20 - DNA, 27 bp, Artificial sequence
  Synthetic oligonucleotide
catgcccatgaacacataccctttgca

SEQ ID NO: 21 - DNA, 23 bp, Artificial sequence
  Synthetic oligonucleotide
gcaagatcaagaagctcgctgta

SEQ ID NO: 22 - DNA, 21 bp, Artificial sequence
  Synthetic oligonucleotide
actcgccggaaaaacatcttt

SEQ ID NO: 23 - DNA, 26 bp, Artificial sequence
  Synthetic oligonucleotide
cgagccgatgaacacataccctttgc

SEQ ID NO: 24 - DNA, 23 bp, Artificial sequence
  Synthetic oligonucleotide
gacgtaccatggctaaaaagcaa

SEQ ID NO: 25 - DNA, 20 bp, Artificial sequence
  Synthetic oligonucleotide
cgatggatttcctcgcaact

SEQ ID NO: 26 - DNA, 21 bp, Artificial sequence
  Synthetic oligonucleotide
ccagtcccacgtgcacccagg

SEQ ID NO: 27 - DNA, 19 bp, Artificial sequence
  Synthetic oligonucleotide
gctgcaacagacccggtta

SEQ ID NO: 28 - DNA, 19 bp, Artificial sequence
  Synthetic oligonucleotide
ctggcgggtccttctgatt

SEQ ID NO: 29 - DNA, 29 bp, Artificial sequence
  Synthetic oligonucleotide
ccgaagaggaacaacacaaaggacttccc

SEQ ID NO: 30 - DNA, 26 bp, Artificial sequence
  Synthetic oligonucleotide
ttgtcttgaattttagctttgacgtt

SEQ ID NO: 31 - DNA, 21 bp, Artificial sequence
  Synthetic oligonucleotide
ccttgaccggaaaaacaatca

SEQ ID NO: 32 - DNA, 27 bp, Artificial sequence
  Synthetic oligonucleotide
tcaatggtgtcggagctttccacttcc